European Patent Application EP 4 215 214 A1, published July 26, 2023. Title: MEDICINE FOR TREATING CANCER AND METHOD FOR SCREENING ANTICANCER SUBSTANCE. Applicant: Osaka University. The sequence listing filed with the application follows.

SEQUENCE LISTING (2 sequences)

SEQ ID NO: 1 - DNA, 1698 bp, Homo sapiens
ctctgtgccagctagtctgggaagttcctctcccgctctaaccacagcccgaggggggctcccctcccccgacctgcaccggagatctcaggcacccggctcatctcagacctcccgctcccgaccctacacagagattgcctggggaggctgaggagccgatgcaaacccccaaggcgacgcacttgggagccggtggtctcaaacacctgccgggggtcctagtccccttctgaaatctacatgcttgggttggagcgcagcagtaaacaccctgcccagtgacctggactgaggcgcgctgggggtgggtgcgccgtgtggcctgagcaggagccagaccaggaggcctaggggtgagagacacattcccctcgctgctcccaaagccagagcccaggctgggcgcccatgcccagaaccatcaagggatcccttgcggcttgtcagcactttccctaatggaaatacaccattaattcctttccaaatgttttaattgtgagagtatctgatattcttgactgaacaatgtaaaaaacccaaagggggctgcgcacggcggctctcgcctaaatcccagcactttgggaggccgaggtgggcagatcacctgaggtcgggagttcgacaccagcctgaccaacatagagaaaccccgtctctactaaaaatacaaaattagccgggcgtggtggttcatgcctgtaatcccagctactcgggaggcttaggtaggagaatcacttgaacccgggaggcggaggttgtggtgggccaagattgtgccaccgcactccagcctgggtaacaaaagcgaaactccatctcaaaaaaagaaacgcaaacggtgcagctgcccctttttcgaggcacgtccacctcccattacccacttccttttttttttgagactgagtcttgctctgtcccctgggctgtagtggagtggctccatctcggctcactgcagccactcccaacgccctccactcctccctactccgcgctggccggggcggggttccgctggtcgcatccaataataagaacaggcggcgcgcgcccttcccggaaactcccgcctggccaccataaaagcgccggccctccgcttccccgcgagacgaaacttcccgtcccggcggctctggcacccaggtactggggaccccagacccacgcggtgcaggccgggagcgagagcctccgtgggggctccgtgaccccggaggggtagagccaagagctgggggagcctgagagatgagggtcgggcggggagggaggcggaggcggaggcggggttccgcggagctgagaaccggacggggtgggatcgaggagggtgcgaagcgccactgtttaggtttcgctttcccgggagcctgacccgcccctgacgtcgcctttcccgtctccgcagggtccggcctgcgccttcccgccaggcctggacactggttcaacacctgtgacttcatgtgtgcgcgccggccacacctgcagtcacacctgtagccccctctgccaagagatccataccgaggcagcgtcggtggctacaagccctcagtccacacctgtggacacctgtgacacctggccacacgacctgtggccgcggcctggcgtctgctgcgacaggagcccttacctcccctgttataacacctgaccgccacctaactgcccctg

SEQ ID NO: 2 - DNA, 881 bp, Homo sapiens
gcacccctgggtttaagtccacactccccaccaccccggcccccacccccaagcagtgacagactgtcttgaacttctcgctgcaagggtcataaaagggacagagaacagagcgacagaagatgtcttctgcattctcaacttttagccccagttgttagagaactggtatctcccctacacgtctggctctggtggagaaagaatgacagcccctacttacaacgaggagactgtggctcagagaagttagggggctgcccaggatcctggagaaagccagctttgactcataaccctcgcgccattacctgactcccattagtggagtcaggaactccatgttccacttcaggaaatgagcttgttgatttttcatttacacaaaaatgaaaaataaataccagatgtttgaaaacatgttgcaacacgtcctgctggaacttaaaagtgcattctgaccaaaaaaattaaattagaaaatccacatagcaaaaaaaaaaatgttttggatgaaaatatactttatctttctctcacacatactctctctctctctcgcacacatacccacacacacacacacacacacacacgcgcgcgcgaaaacaatatctcatttcttcttcagggagcagctgtgaaggaaatcgggggaggaggatggacacaacatcccatctttgtgtttcgatacagactaagcttttaggccaaccctcctgactggatgggggcggcgggcgtggcatgcatgaaaagtaaacatcagagacctgaagaagcttataaaatagcttgggagaggccagtcaccaagacaggcatctcaaatcggctgattctgcatctggaaactgccttcatcttgaaagaaaagg